European Patent Application EP 4 410 827 A1, published August 7, 2024. Title: GLP-1/GIP双靶多肽、融合蛋白及其应用. Applicant: 广东东阳光药业有限公司. Application CN. The sequence listing filed with the application follows.

SEQUENCE LISTING (122 sequences)

SEQ ID NO: 1 - protein, 10 aa, synthetic construct
GPSSGAPPPS

SEQ ID NO: 2 - protein, 39 aa, synthetic construct
YAEGTFTSDYSIYLDKQAAKEFVNWLLAGGPSSGAPPPS

SEQ ID NO: 3 - protein, 39 aa, synthetic construct
YGEGTFTSDYSIYLDKQAAKEFVNWLLAGGPSSGAPPPS

SEQ ID NO: 4 - protein, 39 aa, synthetic construct
YGEGTFTSDYSIALDKQAAKEFVNWLLAGGPSSGAPPPS

SEQ ID NO: 5 - protein, 39 aa, synthetic construct
YGEGTFTSDYSIYLDKKAQRDFVEWLLAQGPSSGAPPPS

SEQ ID NO: 6 - protein, 39 aa, synthetic construct
YGEGTFTSDYSIALDKIAQKAFVQWLIAGGPSSGAPPPS

SEQ ID NO: 7 - protein, 39 aa, synthetic construct
YGEGTFTSDYSIYLDKIAQKAFVQWLIAGGPSSGAPPPS

SEQ ID NO: 8 - protein, 39 aa, synthetic construct
YGEGTFTSDYSIALDKIAAKAFVQWLIAGGPSSGAPPPS

SEQ ID NO: 9 - protein, 39 aa, synthetic construct
YGEGTFTSDYSIALDKQAAKAFVQWLIAGGPSSGAPPPS

SEQ ID NO: 10 - protein, 39 aa, synthetic construct
YGEGTFTSDYSIALDKQRAKDFVQWLIAGGPSSGAPPPS

SEQ ID NO: 11 - protein, 29 aa, synthetic construct
YSEGTFTSDYSKLLEEEAVRLFIEWLLAG

SEQ ID NO: 12 - protein, 29 aa, synthetic construct
YSEGTFTSDYSKLLEEEAVRLFIEWLVKG

SEQ ID NO: 13 - protein, 39 aa, synthetic construct
YGEGTFTSDYSIYLDKKAQRDFVEWLLAGGPSSGAPPPS

SEQ ID NO: 14 - protein, 39 aa, synthetic construct
YGEGTFTSDYSIYLDKKAQRDFVEWLKAGGPSSGAPPPS

SEQ ID NO: 15 - protein, 39 aa, synthetic construct
YGEGTFTSDYSIYLDKKAQRDFVEWLVKGGPSSGAPPPS

SEQ ID NO: 16 - protein, 39 aa, synthetic construct
YGEGTFTSDYSIYLDKKAQRDFVEWLIAGGPSSGAPPPS

SEQ ID NO: 17 - protein, 39 aa, synthetic construct
YGEGTFTSDYSIALDKKAQRDFVEWLLAQGPSSGAPPPS

SEQ ID NO: 18 - protein, 39 aa, synthetic construct
YGEGTFTSDYSIALDKKAQRDFIEWLLAQGPSSGAPPPS

SEQ ID NO: 19 - protein, 39 aa, synthetic construct
YGEGTFISDYSIYLDKKAQRDFVEWLLAQGPSSGAPPPS

SEQ ID NO: 20 - protein, 39 aa, synthetic construct
YGEGTFTSDYSIYLDKKAQRDFVQWLLAQGPSSGAPPPS

SEQ ID NO: 21 - protein, 39 aa, synthetic construct
YGEGTFTSDYSIYLDKKAQRDFIQWLLAQGPSSGAPPPS

SEQ ID NO: 22 - protein, 39 aa, synthetic construct
YGEGTFTSDYSIYLDKKAQRLFIEWLLAQGPSSGAPPPS

SEQ ID NO: 23 - protein, 39 aa, synthetic construct
YGQGTFTSDYSIYLDKKAQRDFVEWLLAQGPSSGAPPPS

SEQ ID NO: 24 - protein, 29 aa, synthetic construct
YAEGTFTSDYSKLLEEEAVRLFIEWLLAG

SEQ ID NO: 25 - protein, 39 aa, synthetic construct
YGEGTFTSDYSIYLDKQAQRDFVEWLIAGGPSSGAPPPS

SEQ ID NO: 26 - protein, 39 aa, synthetic construct
YAEGTFTSDYSIYLDKLAQQEFIDWLKAGGPSSGAPPPS

SEQ ID NO: 27 - protein, 39 aa, synthetic construct
YAEGTFTSDYSIYLDKLAQQAFIEWLKAGGPSSGAPPPS

SEQ ID NO: 28 - protein, 39 aa, synthetic construct
YAEGTFTSDYSIYLDKLAQQAFIEWLLAGGPSSGAPPPS

SEQ ID NO: 29 - protein, 39 aa, synthetic construct
YAEGTFTSDYSIYLDKIAQQAFIEWLKAGGPSSGAPPPS

SEQ ID NO: 30 - protein, 39 aa, synthetic construct
HGEGTFTSDYSIYLDKIAQQAFIEWLLAGGPSSGAPPPS

SEQ ID NO: 31 - protein, 39 aa, synthetic construct
HGQGTFTSDYSIYLDKIAQQAFIEWLLAGGPSSGAPPPS

SEQ ID NO: 32 - protein, 29 aa, synthetic construct
YGEGTFTSDYSIYLDKKAQRDFVEWLLAG

SEQ ID NO: 33 - protein, 39 aa, synthetic construct
YGEGTFTSDYSIALDKKAQRDFIEWLLAGGPSSGAPPPS

SEQ ID NO: 34 - protein, 29 aa, synthetic construct
YGEGTFTSDYSIYLDKKAQRDFVEWLIAG

SEQ ID NO: 35 - protein, 39 aa, synthetic construct
YGEGTFTSDYSIYLDKKAQRDFIEWLIAGGPSSGAPPPS

SEQ ID NO: 36 - protein, 39 aa, synthetic construct
YGEGTFTSDYSIYLDKQAQRDFVEWLLAGGPSSGAPPPS

SEQ ID NO: 37 - protein, 39 aa, synthetic construct
YAEGTFTSDYSIYLDKIAQQAFIEWLLAGGPSSGAPPPS

SEQ ID NO: 38 - protein, 29 aa, synthetic construct
YGEGTFTSDYSIYLDKQAQRDFVEWLLAG

SEQ ID NO: 39 - protein, 39 aa, synthetic construct
YGEGTFTSDYSIYLDKKAQQDFVEWLIAGGPSSGAPPPS

SEQ ID NO: 40 - protein, 39 aa, synthetic construct
YGEGTFTSDYSIYLDKQAQRAFIEWLIAGGPSSGAPPPS

SEQ ID NO: 41 - protein, 39 aa, synthetic construct
YGEGTFTSDYSIYLDKLAQQDFVEWLIAGGPSSGAPPPS

SEQ ID NO: 42 - protein, 39 aa, synthetic construct
YGEGTFTSDYSIALDKLAQQDFIEWLLAGGPSSGAPPPS

SEQ ID NO: 43 - protein, 39 aa, synthetic construct
YGEGTFTSDYSIALDKKAQQAFIEWLLAGGPSSGAPPPS

SEQ ID NO: 44 - protein, 39 aa, synthetic construct
YGEGTFTSDYSIYLDKLAQQAFIEWLKAGGPSSGAPPPS

SEQ ID NO: 45 - protein, 39 aa, synthetic construct
YGEGTFTSDYSIYLDKLAQQEFIDWLKAGGPSSGAPPPS

SEQ ID NO: 46 - protein, 39 aa, synthetic construct
YGEGTFTSDYSIYLDKIAQQAFIEWLLAGGPSSGAPPPS

SEQ ID NO: 47 - protein, 39 aa, synthetic construct
YGEGTFTSDYSIYLDKLAQRDFVEWLLAGGPSSGAPPPS

SEQ ID NO: 48 - protein, 39 aa, synthetic construct
YGEGTFTSDYSIYLDKKAQQDFVEWLLAGGPSSGAPPPS

SEQ ID NO: 49 - protein, 39 aa, synthetic construct
YGEGTFTSDYSIYLDKKAQQAFVEWLLAGGPSSGAPPPS

SEQ ID NO: 50 - protein, 39 aa, synthetic construct
YGEGTFTSDYSIYLDKLAQQAFVEWLLAGGPSSGAPPPS

SEQ ID NO: 51 - protein, 39 aa, synthetic construct
YSEGTFTSDYSIYLDKKAQRDFVEWLLAGGPSSGAPPPS

SEQ ID NO: 52 - protein, 39 aa, synthetic construct
YGEGTFTSDYSIYLDKKAQRDFVEWLVAGGPSSGAPPPS

SEQ ID NO: 53 - protein, 39 aa, synthetic construct
YGEGTFTSDYSIYLDKLAQQDFVEWLLAGGPSSGAPPPS

SEQ ID NO: 54 - protein, 39 aa, synthetic construct
YGEGTFTSDYSIYLDKKAQREFVEWLLAGGPSSGAPPPS

SEQ ID NO: 55 - protein, 39 aa, synthetic construct
YGEGTFTSDYSIYLDKKAQREFIDWLLAGGPSSGAPPPS

SEQ ID NO: 56 - protein, 39 aa, synthetic construct
YGEGTFTSDYSIYLDKKAQRDFIDWLLAGGPSSGAPPPS

SEQ ID NO: 57 - protein, 39 aa, synthetic construct
YGEGTFTSDYSIYLDKKAQRAFIDWLLAGGPSSGAPPPS

SEQ ID NO: 58 - protein, 39 aa, synthetic construct
YGEGTFTSDYSIYLDKKAQRDFIEWLIAQGPSSGAPPPS

SEQ ID NO: 59 - protein, 39 aa, synthetic construct
YGEGTFTSDYSIYLDKKAQRDFVEWLIAQGPSSGAPPPS

SEQ ID NO: 60 - protein, 39 aa, synthetic construct
YGEGTFTSDYSIYLDKKAQRDFVQWLLAGGPSSGAPPPS

SEQ ID NO: 61 - protein, 39 aa, synthetic construct
YGEGTFTSDYSIILDKKAQRDFVEWLLAGGPSSGAPPPS

SEQ ID NO: 62 - protein, 39 aa, synthetic construct
YGEGTFTSDYSIALDKKAQRDFIEWLIAGGPSSGAPPPS

SEQ ID NO: 63 - protein, 29 aa, synthetic construct
YGEGTFTSDYSIYLDKKAQRDFIEWLLAG

SEQ ID NO: 64 - protein, 29 aa, synthetic construct
YGEGTFTSDYSIYLDKKAQRDFIEYLLAG

SEQ ID NO: 65 - protein, 39 aa, synthetic construct
YGEGTFTSDYSIALDKQAQRDFVEWLIAGGPSSGAPPPS

SEQ ID NO: 66 - protein, 39 aa, synthetic construct
YGEGTFTSDYSIYLDKQAQRDFVEWLLAQGPSSGAPPPS

SEQ ID NO: 67 - protein, 39 aa, synthetic construct
YGEGTFTSDYSIYLDKIAQRDFVEWLIAGGPSSGAPPPS

SEQ ID NO: 68 - protein, 39 aa, synthetic construct
YGEGTFTSDYSIYLDKQHQRDFVEWLIAGGPSSGAPPPS

SEQ ID NO: 69 - protein, 39 aa, synthetic construct
YGEGTFTSDYSIYLDKKAQRDFINWLIAGGPSSGAPPPS

SEQ ID NO: 70 - protein, 39 aa, synthetic construct
YGEGTFTSDYSIYLDKKHQRDFIEWLIAGGPSSGAPPPS

SEQ ID NO: 71 - protein, 39 aa, synthetic construct
YGEGTFTSDYSIYLDKIAQRDFIEWLIAGGPSSGAPPPS

SEQ ID NO: 72 - protein, 39 aa, synthetic construct
YGEGTFTSDYSIYLDKKAQQDFIEWLIAGGPSSGAPPPS

SEQ ID NO: 73 - protein, 39 aa, synthetic construct
YGEGTFTSDYSIALDKQAQRDFVEWLLAGGPSSGAPPPS

SEQ ID NO: 74 - protein, 39 aa, synthetic construct
YGEGTFTSDYSIYLDKQAQQDFVEWLLAGGPSSGAPPPS

SEQ ID NO: 75 - protein, 39 aa, synthetic construct
YGEGTFTSDYSIYLDKIAQRDFVEWLLAGGPSSGAPPPS

SEQ ID NO: 76 - protein, 39 aa, synthetic construct
YGEGTFTSDYSIYLDKQAQRDFVNWLLAGGPSSGAPPPS

SEQ ID NO: 77 - protein, 39 aa, synthetic construct
YGEGTFTSDYSIYLDKIAQQAFVEWLLAGGPSSGAPPPS

SEQ ID NO: 78 - protein, 39 aa, synthetic construct
YGEGTFTSDYSIYMDKLAQQAFVEWLLAGGPSSGAPPPS

SEQ ID NO: 79 - protein, 39 aa, synthetic construct
YGEGTFTSDYSIYLDKLAQQAFVNWLLAGGPSSGAPPPS

SEQ ID NO: 80 - protein, 39 aa, synthetic construct
YSEGTFTSDYSIYLDKIAQRDFVEWLLAGGPSSGAPPPS

SEQ ID NO: 81 - protein, 39 aa, synthetic construct
YSEGTFTSDYSIALDKKAQRDFVEWLLAGGPSSGAPPPS

SEQ ID NO: 82 - protein, 39 aa, synthetic construct
YSEGTFTSDYSIYLDKKAQQDFVEWLLAGGPSSGAPPPS

SEQ ID NO: 83 - protein, 39 aa, synthetic construct
YGEGTFTSDYSIALDKKAQRDFIDWLLAGGPSSGAPPPS

SEQ ID NO: 84 - protein, 39 aa, synthetic construct
YGEGTFTSDYSIYLDKKAQRDFINWLLAGGPSSGAPPPS

SEQ ID NO: 85 - protein, 39 aa, synthetic construct
YGEGTFTSDYSIYLDKKAQQDFIDWLLAGGPSSGAPPPS

SEQ ID NO: 86 - protein, 39 aa, synthetic construct
YGEGTFTSDYSIYLDKKAQRDFINWLIAQGPSSGAPPPS

SEQ ID NO: 87 - protein, 39 aa, synthetic construct
YGEGTFTSDYSIALDKKAQRDFIEWLIAQGPSSGAPPPS

SEQ ID NO: 88 - protein, 39 aa, synthetic construct
YGEGTFTSDYSIYLDKKAQQDFIEWLIAQGPSSGAPPPS

SEQ ID NO: 89 - protein, 39 aa, synthetic construct
YGEGTFTSDYSIYLDKIAQRDFIEWLIAQGPSSGAPPPS

SEQ ID NO: 90 - protein, 39 aa, synthetic construct
YGEGTFTSDYSILLDKKAQRDFVEWLLAGGPSSGAPPPS

SEQ ID NO: 91 - protein, 39 aa, synthetic construct
YGEGTFTSDYSIYLDKKAQHDFVEWLLAGGPSSGAPPPS

SEQ ID NO: 92 - protein, 39 aa, synthetic construct
YGEGTFTSDYSIYLDKQAQHAFIEWLIAGGPSSGAPPPS

SEQ ID NO: 93 - protein, 39 aa, synthetic construct
HSEGTFTSDYSILLDKIAQQDFVEWLLAGGPSSGAPPPS

SEQ ID NO: 94 - protein, 39 aa, synthetic construct
HSEGTFTSDYSILLDKIAQHDFIEWLIAGGPSSGAPPPS

SEQ ID NO: 95 - protein, 39 aa, synthetic construct
YSEGTFTSDYSILLDKIAQREFIEWLLAGGPSSGAPPPS

SEQ ID NO: 96 - protein, 39 aa, synthetic construct
HSEGTFTSDYSILLDKIAQREFIEWLLAGGPSSGAPPPS

SEQ ID NO: 97 - protein, 39 aa, synthetic construct
HSEGTFTSDYSILLDKIAQREFIEWLLEGGPSSGAPPPS

SEQ ID NO: 98 - protein, 39 aa, synthetic construct
HSEGTFTSDYSILLDKIAQKEFIEWLLAGGPSSGAPPPS

SEQ ID NO: 99 - protein, 39 aa, synthetic construct
YSEGTFTSDYSILLDKIAQKEFIEWLLAGGPSSGAPPPS

SEQ ID NO: 100 - protein, 39 aa, synthetic construct
HSEGTFTSDYSILLDKIAQKEFIEWLLEGGPSSGAPPPS

SEQ ID NO: 101 - protein, 39 aa, synthetic construct
YSEGTFTSDYSILLDKIAQRAFIEWLLAGGPSSGAPPPS

SEQ ID NO: 102 - protein, 39 aa, synthetic construct
YSEGTFTSDYSILLDKIAQREFIEWLIAGGPSSGAPPPS

SEQ ID NO: 103 - protein, 39 aa, synthetic construct
YSEGTFTSDYSILLDKIAQREFVQWLLAGGPSSGAPPPS

SEQ ID NO: 104 - protein, 39 aa, synthetic construct
YSEGTFTSDYSILLDKIAQREFVQWLIAGGPSSGAPPPS

SEQ ID NO: 105 - protein, 39 aa, synthetic construct
YSEGTFTSDYSILLDKIAQRAFVQWLIAGGPSSGAPPPS

SEQ ID NO: 106 - protein, 39 aa, synthetic construct
YGEGTFTSDYSILLDKIAQREFIEWLLAGGPSSGAPPPS

SEQ ID NO: 107 - protein, 39 aa, synthetic construct
YSEGTFTSDYSILLDKKAQRDFIEWLLAGGPSSGAPPPS

SEQ ID NO: 108 - protein, 39 aa, synthetic construct
YGEGTFTSDYSILLDKKAQRDFIEWLLAGGPSSGAPPPS

SEQ ID NO: 109 - protein, 39 aa, synthetic construct
YSEGTFTSDYSILLDKKAQRDFIEWLIAGGPSSGAPPPS

SEQ ID NO: 110 - protein, 39 aa, synthetic construct
YSEGTFTSDYSILLDKKAQRDFVQWLIAGGPSSGAPPPS

SEQ ID NO: 111 - protein, 39 aa, synthetic construct
YSEGTFTSDYSILLDKIAQRDFVEWLIAGGPSSGAPPPS

SEQ ID NO: 112 - protein, 39 aa, synthetic construct
YGEGTFTSDYSILLDKIAQRDFVEWLIAGGPSSGAPPPS

SEQ ID NO: 113 - protein, 684 aa, synthetic construct
GLUSERLYSTYRGLYPROPROCYSPROPROCYSPROALAPROGLUALAALAGLYGLYPROSERVALPHELEUPHEPROPROLYSPROLYSASPTHRLEUMETILESERARGTHRPROGLUVALTHRCYSVALVALVALASPVALSERGLNGLUASPPROGLUVALGLNPHEASNTRPTYRVALASPGLYVALGLUVALHISASNALALYSTHRLYSPROARGGLUGLUGLNPHEASNSERTHRTYRARGVALVALSERVALLEUTHRVALLEUHISGLNASPTRPLEUASNGLYLYSGLUTYRLYSCYSLYSVALSERASNLYSGLYLEUPROSERSERILEGLULYSTHRILESERLYSALALYSGLYGLNPROARGGLUPROGLNVALTYRTHRLEUPROPROSERGLNGLUGLUMETTHRLYSASNGLNVALSERLEUTHRCYSLEUVALLYSGLYPHETYRPROSERASPILEALAVALGLUTRPGLUSERASNGLYGLNPROGLUASNASNTYRLYSTHRTHRPROPROVALLEUASPSERASPGLYSERPHEPHELEUTYRSERARGLEUTHRVALASPLYSSERARGTRPGLNGLUGLYASNVALPHESERCYSSERVALMETHISGLUALALEUHISASNHISTYRTHRGLNLYSSERLEUSERLEUSERLEUGLY

SEQ ID NO: 114 - protein, 48 aa, synthetic construct
GLYGLYGLYGLYSERGLYGLYGLYGLYSERGLYGLYGLYGLYSERALA

SEQ ID NO: 115 - protein, 31 aa, synthetic construct
HAEGTFTSDVSSYLEGQAAKEFIAWLVKGRG

SEQ ID NO: 116 - protein, 29 aa, synthetic construct
YAEGTFISDYSIAMDKIHQQDFVNWLLAQ

SEQ ID NO: 117 - protein, 39 aa, synthetic construct
YSEGTFTSDYSILLDKIAQQDFVEWLLAGGPSSGAPPPS

SEQ ID NO: 118 - protein, 39 aa, synthetic construct
YSEGTFTSDYSILLDKIAQQEFIEWLLAGGPSSGAPPPS

SEQ ID NO: 119 - protein, 39 aa, synthetic construct
YSEGTFTSDYSILLDKIAQQEFIEWLIAGGPSSGAPPPS

SEQ ID NO: 120 - protein, 39 aa, synthetic construct
YSEGTFTSDYSILLDKKAQQDFIEWLLAGGPSSGAPPPS

SEQ ID NO: 121 - protein, 39 aa, synthetic construct
YSEGTFTSDYSILLDKKAQQDFIEWLIAGGPSSGAPPPS

SEQ ID NO: 122 - protein, 29 aa, synthetic construct
YAEGTFISDYSIAMDKIHQQDFVNWLLAQ